European Patent Application EP 4 137 500 A1, published February 22, 2023. Title: METHOD FOR PRODUCING NUCLEIC ACID OLIGOMER. Applicant: SUMITOMO CHEMICAL COMPANY, LIMITED. The sequence listing filed with the application follows.

SEQUENCE LISTING (2 sequences)

SEQ ID NO: 1 - RNA, 103 nt, Artificial Sequence
  Synthetic oligonucleotide
auaacucaauuuguaaaaaaguuuuagagcuagaaauagcaaguuaaaauaaggcuaguccguuaucaacuugaaaaaguggcaccgagucggugcuuuuuuu

SEQ ID NO: 2 - RNA, 67 nt, Artificial Sequence
  Synthetic oligonucleotide
  modified_base (4)..(4), (6)..(6), (14)..(14), (25)..(25), (37)..(37), (42)..(46): am
  modified_base (2)..(2), (7)..(7), (22)..(22), (41)..(41), (47)..(47), (55)..(55),(61)..(61), (63)..(63): gm
  modified_base (29)..(29), (38)..(38), (53)..(54): cm
  modified_base (5)..(5), (39)..(40), (48)..(48), (62)..(62): um
  modified_base (23)..(23), (28)..(28): phosphorothioate derivative of cytosine
  modified_base (24)..(24), (27)..(27): phosphorothioate derivative of uracil
  modified_base (26)..(26): phosphorothioate derivative of guanine
  modified_base (1)..(1): phosphorothioate derivative of 2'-O-methyladenosine
  modified_base (2)..(2): phosphorothioate derivative of 2'-O-methyllguanosine
  modified_base (3)..(3), (64)..(64): phosphorothioate derivative of 2'-O-methyllcytidine
  modified_base (65)..(66): phosphorothioate derivative of 2'-O-methylluridine
nnnnnnncaaguunaaauaagnnnnnnnnguuaucannnnnnnnnnnnggcannnagucgnnnnnnu